European Patent Application EP 4 534 693 A1, published April 9, 2025. Title: USE OF CIRCULAR RNA IN PREPARING CEREBRAL STROKE DIAGNOSTIC PRODUCTS. Applicant: SHENZHEN HONGJI BIOTECHNOLOGY CO., LTD. The sequence listing filed with the application follows.

SEQUENCE LISTING (6 sequences)

SEQ ID NO: 1 - RNA, 327 nt, synthetic construct
  source 1..327: mol_type = other RNA
gcacaacccgatctcccagagaaggagaagtgcctggcgtggactataactttctgactgtgaaggagttcttggacctcgagcagagtgggactcttctggaagtcggcacctatgaaggaaactattatgggacacccaagcctcctagccagccagtcagtgggaaagtgatcacgacggatgccttgcacagccttcagtctggctctaagcagtcgaccccgaagcgaaccaagtcctacaatgatatgcaaaatgctggcatagtccacgcggagaatgaggaggaggatgacgttcctgaaatgaacagcagctttacag

SEQ ID NO: 2 - DNA, 20 bp, synthetic construct
  source 1..20: mol_type = other DNA
tctgctcgaggtccaagaac

SEQ ID NO: 3 - DNA, 22 bp, synthetic construct
  source 1..22: mol_type = other DNA
cagcagctttacaggcacaacc

SEQ ID NO: 4 - RNA, 327 nt, synthetic construct
  source 1..327: mol_type = other RNA
gcacaacccggtctcccagagaaggagaagtgcctggtgtggattacagctttctgactgtgaaggagttcttggacctcgagcagagcgggaccctgttggaagtcggcacctatgaaggaaactattatgggacacccaaacctcctagccagccagtcagtgggaaagtgatcacgacggatgccttgcacagcctgcagtctggctccaagcagtcgacccctaagcgaacaaagtcctacaatgatatgcaaaatgctggcatagtccacccggagaatgaggaggaggaggatgtccctgaaatgaacagtagctttacag

SEQ ID NO: 5 - DNA, 20 bp, synthetic construct
  source 1..20: mol_type = other DNA
tctgctcgaggtccaagaac

SEQ ID NO: 6 - DNA, 22 bp, synthetic construct
  source 1..22: mol_type = other DNA
cagtagctttacaggcacaacc